European Patent Application EP 4 393 508 A1, published July 3, 2024. Title: A composition for suppressing transdifferentiation of mature hepatocyte. Applicant: Osaka University. Application WO. The sequence listing filed with the application follows.

SEQUENCE LISTING (11 sequences)

SEQ ID NO: 1 - RNA, 57 nt, synthetic construct
  modified_base 6: mod_base = OTHER; note = thymine
  modified_base 13: mod_base = OTHER; note = thymine
  modified_base 18: mod_base = OTHER; note = thymine
  modified_base 23..24: mod_base = OTHER; note = thymine
  modified_base 27: mod_base = OTHER; note = thymine
  modified_base 32: mod_base = OTHER; note = thymine
  modified_base 35: mod_base = OTHER; note = thymine
  modified_base 38: mod_base = OTHER; note = thymine
  modified_base 42: mod_base = OTHER; note = thymine
  modified_base 46: mod_base = OTHER; note = thymine
  modified_base 49: mod_base = OTHER; note = thymine
  modified_base 53..57: mod_base = OTHER; note = thymine
  misc_feature 1..57: note = MAP3K14 shRNA
  source 1..57: mol_type = other RNA
ccggctcaggactcacgtagcattactcgagtaatgctacgtgagtcctgagttttt

SEQ ID NO: 2 - RNA, 21 nt, synthetic construct
  modified_base 20..21: mod_base = OTHER; note = thymine
  misc_feature 1..21: note = MAP3K14 siRNA
  source 1..21: mol_type = other RNA
caaacgcaaagagcaagaatt

SEQ ID NO: 3 - RNA, 21 nt, synthetic construct
  misc_feature 1..21: note = MAP3K14 siRNA
  source 1..21: mol_type = other RNA
ttcttgctctttgcgtttgca

SEQ ID NO: 4 - RNA, 21 nt, synthetic construct
  modified_base 20..21: mod_base = OTHER; note = thymine
  misc_feature 1..21: note = MAP3K14 siRNA
  source 1..21: mol_type = other RNA
gcaaagagcaagaaccaaatt

SEQ ID NO: 5 - RNA, 21 nt, synthetic construct
  modified_base 21: mod_base = OTHER; note = thymine
  misc_feature 1..21: note = MAP3K14 siRNA
  source 1..21: mol_type = other RNA
tttggttcttgctctttgcgt

SEQ ID NO: 6 - RNA, 21 nt, synthetic construct
  modified_base 20..21: mod_base = OTHER; note = thymine
  misc_feature 1..21: note = Traf3 siRNA
  source 1..21: mol_type = other RNA
ggataattgctgcaagagatt

SEQ ID NO: 7 - RNA, 21 nt, synthetic construct
  modified_base 20..21: mod_base = OTHER; note = thymine
  misc_feature 1..21: note = Traf3 siRNA
  source 1..21: mol_type = other RNA
tctcttgcagcaattatcctt

SEQ ID NO: 8 - RNA, 21 nt, synthetic construct
  modified_base 20..21: mod_base = OTHER; note = thymine
  misc_feature 1..21: note = Pten siRNA
  source 1..21: mol_type = other RNA
gcatacgattttaagcggatt

SEQ ID NO: 9 - RNA, 21 nt, synthetic construct
  misc_feature 1..21: note = Pten siRNA
  source 1..21: mol_type = other RNA
tccgcttaaaatcgtatgcag

SEQ ID NO: 10 - RNA, 21 nt, synthetic construct
  modified_base 20..21: mod_base = OTHER; note = thymine
  misc_feature 1..21: note = Pten siRNA
  source 1..21: mol_type = other RNA
ggttttcgagtcctaattatt

SEQ ID NO: 11 - RNA, 21 nt, synthetic construct
  misc_feature 1..21: note = Pten siRNA
  source 1..21: mol_type = other RNA
  modified_base 20..21: mod_base = OTHER; note = thymine
taattaggactcgaaaacctt